European Patent Application EP 4 279 604 A2, published November 22, 2023. Title: MODIFIED BETA-GALACTOSIDASE. Applicant: AMANO ENZYME INC. The sequence listing filed with the application follows.

SEQUENCE LISTING (33 sequences)

SEQ ID NO: 1 - protein, 1737 aa, Bacillus circulans
MKKAISCVFLISALILSSFQVPVQGQAMSKTTSAAGNSVSYDGERRVNFNENWRFQRETNGSIAGAQNPGFDDSSWRKLNLPHDWSIELDFNKNSLATHEGGYLDGGIGWYRKTFTIPESMKGKRISLDFDGVYMNSTTYLNGEVLGTYPFGYNAFSYDISDKLYKDGRANVLVVKVNNTQPSSRWYSGSGIYRNVYLTVTDPIHVARYGTFVTTPNLEKSIKEDRADVNIKTKISNDAAEAKQVKIKSTIYDGAGNTVQTVETEEKTAAAGTVTPFEQNTVIKQPKLWSIDKPYRYNLVTEVIVGGQTVDTYETKFGVRYFKFDENEGFSLNGEYMKLHGVSMHHDLGALGAATNARGVERQMQIMKDMGVNAIRVTHNPASPELLEAANKLGLFIIEEAFDSWAQSKKPYDYGRFFNAWAEHDIKEMVDRGKNEPAIIMWSIGNEIYDTTNAAGVETARNLVGWVKEIDTTRPTTIGEDKTRGDKVNVTPINSYIKEIFNIVDVVGLNYSENNYDGYHKQNPSWKLYGSETSSATRSRGVYTHPYQYNQSTKYADLQQSSYDNDYVGWGRTAEDAWKYDRDLKHIAGQFIWTGFDYIGEPTPYYNSYPAKSSYFGAVDTAGFPKDIFYYYQSQWKKEPMVHLLPHWNWKEGEKVRVLAYTNASKVELVLNGESLGEKNYDNKQTSWGAPYKETKDGKTYLEWAVPFKPGKLEAVAKDENGKVIARDQVVTAGEPASVRLTADRKVVKADGTDLSFITADIVDSKGIVVPDADHLITFNVTGQGELAGVDNGNASSVERYKDNKRKAFSGKALAIVQSSKLSGKITVHASVAGLSSDSTSVFTVTPADHDKKIVAGIDDVNLTVDVNEAPKLPSEIKVYYSDESAAAKNVTWDEVDPKQYSTVGEFTVEGSVEGTSLKAKAFVIVKGIVAVKPYSTATKVGVQPVLPEKATLLYSDGTTKGATVTWDEIPEDKLAKEGRFTVEGSVEGTDLKANVYVRVTNEVKSVNIMLQEQGSAYPKLEATFTNPADNLQHLNDGIKSYTNNPVNRWTNWTRTPRDAGDSITVNFGKKHVINNLDLFVFTDSGTVVPEKAEVQYWDGTAWKDVENLTQPSPYVVEKNELTFDAVATEKLKFHLTPSVKGKFLALTEAEVYADQIVMGETAKLQSITVNGKALEGFDHAKKNYELVLPYGSELPKIEAAAADNATVTILPAFSYPGTAKLFVTSEDGKVTTEYSIGVSTEEPKLVSAELSADKTNVMEDDIIDLKVIGLFESKEKIDVTDSQPTYEFDQQIIKIEGNKLYALETGNVKVKVTVTYKGVSVTTPALEFTIAKNPAPKYITSLEPVTVVVKKGEAPELPATVVAHYNRGIPRDVKVKWERINPSKYQQLGEFTVSGMVEGTDIKAQAKVIVKGAVAVEDIRMAVLLKQMPQLPGKVTVYYSDGAEEQRAVKWEEIPQEELENVGEFKVKGDVNGVKLKATATIRVTDEVGGEQNISRAKNGYEYPKAEASFTNNGPGSSDRIEAINDDVISYEANPHNRWTNWQPVPRAGDWVSITFGDYEPTEYDVDSMEIHWFADHGTSYPERFQIEYKSGDSWKEVTSLKSDPASPALGKANVYSFDRVKTSAIRVKMTAQAGKSLAITELKVFSKWPKAGTEPEVTDIKVGGKSILEDFEQKGDHYEVTIDAGDANVMPKINVKAKDQTSITIVPAVTSPSTAKVIAKSEDGKKVKVYSIHYK

SEQ ID NO: 2 - protein, 1422 aa, Bacillus circulans
MKKAISCVFLISALILSSFQVPVQGQAMSKTTSAAGNSVSYDGERRVNFNENWRFQRETNGSIAGAQNPGFDDSSWRKLNLPHDWSIELDFNKNSLATHEGGYLDGGIGWYRKTFTIPESMKGKRISLDFDGVYMNSTTYLNGEVLGTYPFGYNAFSYDISDKLYKDGRANVLVVKVNNTQPSSRWYSGSGIYRNVYLTVTDPIHVARYGTFVTTPNLEKSIKEDRADVNIKTKISNDAAEAKQVKIKSTIYDGAGNTVQTVETEEKTAAAGTVTPFEQNTVIKQPKLWSIDKPYRYNLVTEVIVGGQTVDTYETKFGVRYFKFDENEGFSLNGEYMKLHGVSMHHDLGALGAATNARGVERQMQIMKDMGVNAIRVTHNPASPELLEAANKLGLFIIEEAFDSWAQSKKPYDYGRFFNAWAEHDIKEMVDRGKNEPAIIMWSIGNEIYDTTNAAGVETARNLVGWVKEIDTTRPTTIGEDKTRGDKVNVTPINSYIKEIFNIVDVVGLNYSENNYDGYHKQNPSWKLYGSETSSATRSRGVYTHPYQYNQSTKYADLQQSSYDNDYVGWGRTAEDAWKYDRDLKHIAGQFIWTGFDYIGEPTPYYNSYPAKSSYFGAVDTAGFPKDIFYYYQSQWKKEPMVHLLPHWNWKEGEKVRVLAYTNASKVELVLNGESLGEKNYDNKQTSWGAPYKETKDGKTYLEWAVPFKPGKLEAVAKDENGKVIARDQVVTAGEPASVRLTADRKVVKADGTDLSFITADIVDSKGIVVPDADHLITFNVTGQGELAGVDNGNASSVERYKDNKRKAFSGKALAIVQSSKLSGKITVHASVAGLSSDSTSVFTVTPADHDKKIVAGIDDVNLTVDVNEAPKLPSEIKVYYSDESAAAKNVTWDEVDPKQYSTVGEFTVEGSVEGTSLKAKAFVIVKGIVAVKPYSTATKVGVQPVLPEKATLLYSDGTTKGATVTWDEIPEDKLAKEGRFTVEGSVEGTDLKANVYVRVTNEVKSVNIMLQEQGSAYPKLEATFTNPADNLQHLNDGIKSYTNNPVNRWTNWTRTPRDAGDSITVNFGKKHVINNLDLFVFTDSGTVVPEKAEVQYWDGTAWKDVENLTQPSPYVVEKNELTFDAVATEKLKFHLTPSVKGKFLALTEAEVYADQIVMGETAKLQSITVNGKALEGFDHAKKNYELVLPYGSELPKIEAAAADNATVTILPAFSYPGTAKLFVTSEDGKVTTEYSIGVSTEEPKLVSAELSADKTNVMEDDIIDLKVIGLFESKEKIDVTDSQPTYEFDQQIIKIEGNKLYALETGNVKVKVTVTYKGVSVTTPALEFTIAKNPAPKYITSLEPVTVVVKKGEAPELPATVVAHYNRGIPRDVKVKWERINPSKYQQLGEFTVSGMVEGTDIKAQAKVIVKGAVAVEDIRM

SEQ ID NO: 3 - protein, 1249 aa, Bacillus circulans
MKKAISCVFLISALILSSFQVPVQGQAMSKTTSAAGNSVSYDGERRVNFNENWRFQRETNGSIAGAQNPGFDDSSWRKLNLPHDWSIELDFNKNSLATHEGGYLDGGIGWYRKTFTIPESMKGKRISLDFDGVYMNSTTYLNGEVLGTYPFGYNAFSYDISDKLYKDGRANVLVVKVNNTQPSSRWYSGSGIYRNVYLTVTDPIHVARYGTFVTTPNLEKSIKEDRADVNIKTKISNDAAEAKQVKIKSTIYDGAGNTVQTVETEEKTAAAGTVTPFEQNTVIKQPKLWSIDKPYRYNLVTEVIVGGQTVDTYETKFGVRYFKFDENEGFSLNGEYMKLHGVSMHHDLGALGAATNARGVERQMQIMKDMGVNAIRVTHNPASPELLEAANKLGLFIIEEAFDSWAQSKKPYDYGRFFNAWAEHDIKEMVDRGKNEPAIIMWSIGNEIYDTTNAAGVETARNLVGWVKEIDTTRPTTIGEDKTRGDKVNVTPINSYIKEIFNIVDVVGLNYSENNYDGYHKQNPSWKLYGSETSSATRSRGVYTHPYQYNQSTKYADLQQSSYDNDYVGWGRTAEDAWKYDRDLKHIAGQFIWTGFDYIGEPTPYYNSYPAKSSYFGAVDTAGFPKDIFYYYQSQWKKEPMVHLLPHWNWKEGEKVRVLAYTNASKVELVLNGESLGEKNYDNKQTSWGAPYKETKDGKTYLEWAVPFKPGKLEAVAKDENGKVIARDQVVTAGEPASVRLTADRKVVKADGTDLSFITADIVDSKGIVVPDADHLITFNVTGQGELAGVDNGNASSVERYKDNKRKAFSGKALAIVQSSKLSGKITVHASVAGLSSDSTSVFTVTPADHDKKIVAGIDDVNLTVDVNEAPKLPSEIKVYYSDESAAAKNVTWDEVDPKQYSTVGEFTVEGSVEGTSLKAKAFVIVKGIVAVKPYSTATKVGVQPVLPEKATLLYSDGTTKGATVTWDEIPEDKLAKEGRFTVEGSVEGTDLKANVYVRVTNEVKSVNIMLQEQGSAYPKLEATFTNPADNLQHLNDGIKSYTNNPVNRWTNWTRTPRDAGDSITVNFGKKHVINNLDLFVFTDSGTVVPEKAEVQYWDGTAWKDVENLTQPSPYVVEKNELTFDAVATEKLKFHLTPSVKGKFLALTEAEVYADQIVMGETAKLQSITVNGKALEGFDHAKKNYELVLPYGSELPKIEAAAADNATVTILPAFSYPGTAKLFVTSEDGKVTTEYSIGVSTEEPKLVSA

SEQ ID NO: 4 - protein, 847 aa, Bacillus circulans
MKKAISCVFLISALILSSFQVPVQGQAMSKTTSAAGNSVSYDGERRVNFNENWRFQRETNGSIAGAQNPGFDDSSWRKLNLPHDWSIELDFNKNSLATHEGGYLDGGIGWYRKTFTIPESMKGKRISLDFDGVYMNSTTYLNGEVLGTYPFGYNAFSYDISDKLYKDGRANVLVVKVNNTQPSSRWYSGSGIYRNVYLTVTDPIHVARYGTFVTTPNLEKSIKEDRADVNIKTKISNDAAEAKQVKIKSTIYDGAGNTVQTVETEEKTAAAGTVTPFEQNTVIKQPKLWSIDKPYRYNLVTEVIVGGQTVDTYETKFGVRYFKFDENEGFSLNGEYMKLHGVSMHHDLGALGAATNARGVERQMQIMKDMGVNAIRVTHNPASPELLEAANKLGLFIIEEAFDSWAQSKKPYDYGRFFNAWAEHDIKEMVDRGKNEPAIIMWSIGNEIYDTTNAAGVETARNLVGWVKEIDTTRPTTIGEDKTRGDKVNVTPINSYIKEIFNIVDVVGLNYSENNYDGYHKQNPSWKLYGSETSSATRSRGVYTHPYQYNQSTKYADLQQSSYDNDYVGWGRTAEDAWKYDRDLKHIAGQFIWTGFDYIGEPTPYYNSYPAKSSYFGAVDTAGFPKDIFYYYQSQWKKEPMVHLLPHWNWKEGEKVRVLAYTNASKVELVLNGESLGEKNYDNKQTSWGAPYKETKDGKTYLEWAVPFKPGKLEAVAKDENGKVIARDQVVTAGEPASVRLTADRKVVKADGTDLSFITADIVDSKGIVVPDADHLITFNVTGQGELAGVDNGNASSVERYKDNKRKAFSGKALAIVQSSKLSGKITVHASVAGLSSDSTSVFTVTP

SEQ ID NO: 5 - DNA, 5214 bp, Bacillus circulans
  source 1..5214: mol_type = genomic DNA
gtgaaaaaagcgattagctgcgtttttttaatttcagcactgattctatcaagctttcaagtccctgtacagggacaagccatgtcaaaaacgacatcggcagcaggaaacagtgtgagctatgatggagagagacgagtgaattttaacgagaattggcgatttcaacgagaaaccaatggaagtattgccggagcacagaatcctggctttgacgattcctcctggcggaaattaaatctgccgcatgactggagtattgaattagattttaataaaaattctcttgccacacatgaaggcggttatttggacggcggaatcggctggtaccgaaaaacctttacaatcccggaatcgatgaagggaaaacgaatttcgcttgattttgatggcgtttacatgaacagcaccacctatctaaacggggaagtgctcgggacctatccgtttggttataatgccttttcctatgatatttccgacaaactttataaagatggcagggcgaatgtccttgttgtcaaagtcaataacacccagccgagcagccgctggtattcggggagcgggatctaccggaatgtctatctcactgtgaccgatcccatccatgtggctcgctacggaacatttgtgacaacacccaatttagagaaatcgataaaagaagacagggctgatgtgaacatcaagacgaaaatcagtaacgatgctgctgaggcgaaacaggtaaagattaaatcaaccatctacgatggggctgggaacaccgtacagacagtggaaacggaggaaaaaacagctgccgccggcacggtgactccgttcgaacaaaacacagtcatcaagcagccgaagctttggagcattgacaagccttatcgatataaccttgttacagaagtcatcgttggcgggcaaacggtggatacgtatgaaacaaaatttggtgtcaggtatttcaaatttgatgaaaacgaaggcttttccttaaatggagagtatatgaagctgcacggcgtttcgatgcaccatgatttaggggcgcttggggcggcaacgaatgcacgcggcgtggaaagacaaatgcagattatgaaggatatgggggtcaatgccatcagggttacccacaacccggcatcaccggaactgctggaggcagctaataaattagggctattcatcatcgaggaggcatttgacagctgggcccagtcaaagaaaccctatgactatggccgttttttcaatgcatgggctgagcacgacattaaggaaatggtcgatcggggcaaaaacgaaccagctattatcatgtggtcgatcggaaatgaaatatatgatacgaccaatgccgctggtgtggaaacagcacgaaatttagtgggttgggtaaaagaaattgacaccacaaggccgacaacgatcggcgaggataaaacccgcggagacaaagtaaatgttacacctatcaacagctacatcaaggagatttttaatattgtcgatgtggtcggactgaactacagcgagaacaactatgatggctaccacaagcagaatccgtcatggaagctgtacggctcggagacgtcctcggcaacccgttcgcgtggtgtctacacgcatccgtaccagtataaccaaagcacaaagtatgctgatttacagcaatcctcttatgacaatgactatgtcggctggggacgaactgcagaagatgcatggaaatatgaccgcgacctgaagcatattgcagggcaatttatctggaccggctttgattatattggcgagccgacgccatattataattcctatcctgcaaaaagctcctattttggtgctgtggatacggctggttttccaaaggatattttctactattaccaaagccaatggaaaaaggagcctatggtccacctgctgccgcattggaactggaaggaaggggaaaaggtccgcgtcttagcttataccaatgcaagtaaggttgaacttgttctaaatggtgaatcgttaggggagaagaactatgacaacaaacaaacctcctggggagcaccatacaaagaaacaaaggatggaaaaacctatttggagtgggccgtaccatttaaaccgggcaaattagaagccgtcgccaaggatgaaaacggcaaagtgatcgcccgcgatcaggtagtgaccgctggtgagccagcctctgtcagattaacggctgatcgtaaggtggtcaaggcggacggtacggatctgtcgtttattacagcagacattgttgatagtaaagggattgttgtcccggatgccgatcatctgattacatttaacgtaacgggccaaggggaattggccggggttgataacggaaacgcgtccagtgtggagcgttacaaggacaacaagcgcaaggctttcagcgggaaagcattggcgattgttcaatcaagtaagctttctggaaaaattacggtccatgcgtcagtggcagggctttcgagcgattccacgagcgtatttacggtaacgccagctgaccatgacaaaaagattgtagctgggattgatgatgttaaccttactgtcgatgtcaatgaagcaccaaagcttccttcagaaatcaaggtttattacagtgatgagagtgcagctgcgaagaatgtgacttgggatgaggtggatccaaagcagtacagcactgttggtgaattcacagtggaaggcagtgtcgagggaacttcgctgaaggcaaaggcatttgttattgtcaaaggaattgtcgccgtcaagccttattcaacggcaacaaaggttggtgtacagccggtgctgcctgaaaaagcaacccttctttacagtgatggaacaaccaagggagcaactgtcacgtgggatgagatccctgaggacaagctggcaaaagagggccggtttaccgtcgagggcagtgtggagggaacagacctcaaggctaatgtctatgtcagggtgacaaatgaagtaaaatcagtgaatattatgcttcaggagcagggttcagcttatccaaagctcgaagctacttttaccaatccagctgacaatcttcagcatttgaacgatggcatcaagagctataccaataacccggtcaaccgctggacgaactggacaagaacaccgcgtgatgctggtgactcgattacagttaattttggcaagaagcatgtgattaataatctagatttatttgtttttaccgacagcggcacggtggttccagaaaaggcagaggtccaatattgggatggaacggcgtggaaggatgtcgaaaatctaacacagccatcgccatatgtggtagagaaaaatgaacttacatttgatgcggtcgcgacagaaaagctgaaattccatttgacaccatctgtgaaagggaaattcctagctctaacggaagcagaggtgtacgccgatcagattgtgatgggtgaaacagcaaaacttcaaagtattacggtgaatgggaaagcattagaaggctttgatcacgctaaaaagaattatgaacttgtacttccatatggaagcgagcttcctaagattgaggcggctgctgccgacaatgcaactgtcaccattttaccggcattctcctatccgggaacagcaaaactatttgtcacttcagaggatgggaaggtaactactgagtacagtattggtgtttctacagaagagccaaagctcgtctccgcagagttatccgcggacaagacgaatgtcatggaggacgatatcatcgatctgaaggtaattggtctcttcgaaagcaaggaaaagattgatgtgaccgacagccagccgacatatgaatttgaccagcagattattaaaattgaaggcaataagctgtatgcgctggaaacaggaaatgtcaaggtgaaagtgacggtgacatataagggtgtgagtgtcacaacacctgcgcttgagtttacgatcgcgaaaaaccctgctccaaaatacattacgagcttagagcctgtcacggttgttgttaaaaaaggagaagcgccggagcttccagcaacggttgtggcccattataaccgaggaatcccgcgggatgttaaggtgaagtgggaaagaatcaatccgtctaagtaccagcagctaggcgagtttaccgtatctggcatggtggaagggaccgatataaaagcccaagcaaaagtgattgtaaaaggggctgttgcggtcgaggatattagaatggctgtgctgttaaagcaaatgccacagctgccgggcaaggttacagtctattatagtgacggagcggaagaacaaagagcggtcaagtgggaggaaatcccgcaggaggaactcgagaatgtcggtgaatttaaggttaaaggtgatgttaatggagtgaagctgaaagcaacagccactattcgagtaaccgatgaagtcggcggcgagcagaatatcagccgggctaaaaatggttatgaatacccgaaggctgaagcttcctttaccaacaatggccctggatcaagcgatcgaatcgaggccatcaatgatgacgtgatctcctacgaggctaatccgcataatcgctggacgaattggcagccggtaccgcgtgcaggggactgggtttctatcacctttggagactatgagcctacggaatatgatgttgatagcatggagatccactggttcgcggatcatgggacctcgtatccagagcgtttccaaatcgaatataaatccggtgatagctggaaggaagtcaccagcctgaaaagcgatccagcctctccggccttgggtaaggcaaatgtctatagctttgatcgagtaaaaacatcggctatacgagtgaaaatgacagcacaagccggcaaaagcttagccattaccgagctgaaagtattttcaaaatggccaaaggcaggtaccgaaccagaggtgaccgatattaaggtcggaggaaaatcgattctggaggactttgaacaaaaaggcgatcactatgaagtaacgattgatgcaggagatgcgaatgtaatgccgaaaatcaatgtaaaggctaaggaccagacgagtattacgattgtgccagcagttacctctccatccacggcaaaggtaattgctaaatccgaggatggcaagaaagtgaaggtctatagcattcactataaataa

SEQ ID NO: 6 - DNA, 4266 bp, Bacillus circulans
  source 1..4266: mol_type = genomic DNA
gtgaaaaaagcgattagctgcgtttttttaatttcagcactgattctatcaagctttcaagtccctgtacagggacaagccatgtcaaaaacgacatcggcagcaggaaacagtgtgagctatgatggagagagacgagtgaattttaacgagaattggcgatttcaacgagaaaccaatggaagtattgccggagcacagaatcctggctttgacgattcctcctggcggaaattaaatctgccgcatgactggagtattgaattagattttaataaaaattctcttgccacacatgaaggcggttatttggacggcggaatcggctggtaccgaaaaacctttacaatcccggaatcgatgaagggaaaacgaatttcgcttgattttgatggcgtttacatgaacagcaccacctatctaaacggggaagtgctcgggacctatccgtttggttataatgccttttcctatgatatttccgacaaactttataaagatggcagggcgaatgtccttgttgtcaaagtcaataacacccagccgagcagccgctggtattcggggagcgggatctaccggaatgtctatctcactgtgaccgatcccatccatgtggctcgctacggaacatttgtgacaacacccaatttagagaaatcgataaaagaagacagggctgatgtgaacatcaagacgaaaatcagtaacgatgctgctgaggcgaaacaggtaaagattaaatcaaccatctacgatggggctgggaacaccgtacagacagtggaaacggaggaaaaaacagctgccgccggcacggtgactccgttcgaacaaaacacagtcatcaagcagccgaagctttggagcattgacaagccttatcgatataaccttgttacagaagtcatcgttggcgggcaaacggtggatacgtatgaaacaaaatttggtgtcaggtatttcaaatttgatgaaaacgaaggcttttccttaaatggagagtatatgaagctgcacggcgtttcgatgcaccatgatttaggggcgcttggggcggcaacgaatgcacgcggcgtggaaagacaaatgcagattatgaaggatatgggggtcaatgccatcagggttacccacaacccggcatcaccggaactgctggaggcagctaataaattagggctattcatcatcgaggaggcatttgacagctgggcccagtcaaagaaaccctatgactatggccgttttttcaatgcatgggctgagcacgacattaaggaaatggtcgatcggggcaaaaacgaaccagctattatcatgtggtcgatcggaaatgaaatatatgatacgaccaatgccgctggtgtggaaacagcacgaaatttagtgggttgggtaaaagaaattgacaccacaaggccgacaacgatcggcgaggataaaacccgcggagacaaagtaaatgttacacctatcaacagctacatcaaggagatttttaatattgtcgatgtggtcggactgaactacagcgagaacaactatgatggctaccacaagcagaatccgtcatggaagctgtacggctcggagacgtcctcggcaacccgttcgcgtggtgtctacacgcatccgtaccagtataaccaaagcacaaagtatgctgatttacagcaatcctcttatgacaatgactatgtcggctggggacgaactgcagaagatgcatggaaatatgaccgcgacctgaagcatattgcagggcaatttatctggaccggctttgattatattggcgagccgacgccatattataattcctatcctgcaaaaagctcctattttggtgctgtggatacggctggttttccaaaggatattttctactattaccaaagccaatggaaaaaggagcctatggtccacctgctgccgcattggaactggaaggaaggggaaaaggtccgcgtcttagcttataccaatgcaagtaaggttgaacttgttctaaatggtgaatcgttaggggagaagaactatgacaacaaacaaacctcctggggagcaccatacaaagaaacaaaggatggaaaaacctatttggagtgggccgtaccatttaaaccgggcaaattagaagccgtcgccaaggatgaaaacggcaaagtgatcgcccgcgatcaggtagtgaccgctggtgagccagcctctgtcagattaacggctgatcgtaaggtggtcaaggcggacggtacggatctgtcgtttattacagcagacattgttgatagtaaagggattgttgtcccggatgccgatcatctgattacatttaacgtaacgggccaaggggaattggccggggttgataacggaaacgcgtccagtgtggagcgttacaaggacaacaagcgcaaggctttcagcgggaaagcattggcgattgttcaatcaagtaagctttctggaaaaattacggtccatgcgtcagtggcagggctttcgagcgattccacgagcgtatttacggtaacgccagctgaccatgacaaaaagattgtagctgggattgatgatgttaaccttactgtcgatgtcaatgaagcaccaaagcttccttcagaaatcaaggtttattacagtgatgagagtgcagctgcgaagaatgtgacttgggatgaggtggatccaaagcagtacagcactgttggtgaattcacagtggaaggcagtgtcgagggaacttcgctgaaggcaaaggcatttgttattgtcaaaggaattgtcgccgtcaagccttattcaacggcaacaaaggttggtgtacagccggtgctgcctgaaaaagcaacccttctttacagtgatggaacaaccaagggagcaactgtcacgtgggatgagatccctgaggacaagctggcaaaagagggccggtttaccgtcgagggcagtgtggagggaacagacctcaaggctaatgtctatgtcagggtgacaaatgaagtaaaatcagtgaatattatgcttcaggagcagggttcagcttatccaaagctcgaagctacttttaccaatccagctgacaatcttcagcatttgaacgatggcatcaagagctataccaataacccggtcaaccgctggacgaactggacaagaacaccgcgtgatgctggtgactcgattacagttaattttggcaagaagcatgtgattaataatctagatttatttgtttttaccgacagcggcacggtggttccagaaaaggcagaggtccaatattgggatggaacggcgtggaaggatgtcgaaaatctaacacagccatcgccatatgtggtagagaaaaatgaacttacatttgatgcggtcgcgacagaaaagctgaaattccatttgacaccatctgtgaaagggaaattcctagctctaacggaagcagaggtgtacgccgatcagattgtgatgggtgaaacagcaaaacttcaaagtattacggtgaatgggaaagcattagaaggctttgatcacgctaaaaagaattatgaacttgtacttccatatggaagcgagcttcctaagattgaggcggctgctgccgacaatgcaactgtcaccattttaccggcattctcctatccgggaacagcaaaactatttgtcacttcagaggatgggaaggtaactactgagtacagtattggtgtttctacagaagagccaaagctcgtctccgcagagttatccgcggacaagacgaatgtcatggaggacgatatcatcgatctgaaggtaattggtctcttcgaaagcaaggaaaagattgatgtgaccgacagccagccgacatatgaatttgaccagcagattattaaaattgaaggcaataagctgtatgcgctggaaacaggaaatgtcaaggtgaaagtgacggtgacatataagggtgtgagtgtcacaacacctgcgcttgagtttacgatcgcgaaaaaccctgctccaaaatacattacgagcttagagcctgtcacggttgttgttaaaaaaggagaagcgccggagcttccagcaacggttgtggcccattataaccgaggaatcccgcgggatgttaaggtgaagtgggaaagaatcaatccgtctaagtaccagcagctaggcgagtttaccgtatctggcatggtggaagggaccgatataaaagcccaagcaaaagtgattgtaaaaggggctgttgcggtcgaggatattagaatg

SEQ ID NO: 7 - DNA, 3747 bp, Bacillus circulans
  source 1..3747: mol_type = genomic DNA
gtgaaaaaagcgattagctgcgtttttttaatttcagcactgattctatcaagctttcaagtccctgtacagggacaagccatgtcaaaaacgacatcggcagcaggaaacagtgtgagctatgatggagagagacgagtgaattttaacgagaattggcgatttcaacgagaaaccaatggaagtattgccggagcacagaatcctggctttgacgattcctcctggcggaaattaaatctgccgcatgactggagtattgaattagattttaataaaaattctcttgccacacatgaaggcggttatttggacggcggaatcggctggtaccgaaaaacctttacaatcccggaatcgatgaagggaaaacgaatttcgcttgattttgatggcgtttacatgaacagcaccacctatctaaacggggaagtgctcgggacctatccgtttggttataatgccttttcctatgatatttccgacaaactttataaagatggcagggcgaatgtccttgttgtcaaagtcaataacacccagccgagcagccgctggtattcggggagcgggatctaccggaatgtctatctcactgtgaccgatcccatccatgtggctcgctacggaacatttgtgacaacacccaatttagagaaatcgataaaagaagacagggctgatgtgaacatcaagacgaaaatcagtaacgatgctgctgaggcgaaacaggtaaagattaaatcaaccatctacgatggggctgggaacaccgtacagacagtggaaacggaggaaaaaacagctgccgccggcacggtgactccgttcgaacaaaacacagtcatcaagcagccgaagctttggagcattgacaagccttatcgatataaccttgttacagaagtcatcgttggcgggcaaacggtggatacgtatgaaacaaaatttggtgtcaggtatttcaaatttgatgaaaacgaaggcttttccttaaatggagagtatatgaagctgcacggcgtttcgatgcaccatgatttaggggcgcttggggcggcaacgaatgcacgcggcgtggaaagacaaatgcagattatgaaggatatgggggtcaatgccatcagggttacccacaacccggcatcaccggaactgctggaggcagctaataaattagggctattcatcatcgaggaggcatttgacagctgggcccagtcaaagaaaccctatgactatggccgttttttcaatgcatgggctgagcacgacattaaggaaatggtcgatcggggcaaaaacgaaccagctattatcatgtggtcgatcggaaatgaaatatatgatacgaccaatgccgctggtgtggaaacagcacgaaatttagtgggttgggtaaaagaaattgacaccacaaggccgacaacgatcggcgaggataaaacccgcggagacaaagtaaatgttacacctatcaacagctacatcaaggagatttttaatattgtcgatgtggtcggactgaactacagcgagaacaactatgatggctaccacaagcagaatccgtcatggaagctgtacggctcggagacgtcctcggcaacccgttcgcgtggtgtctacacgcatccgtaccagtataaccaaagcacaaagtatgctgatttacagcaatcctcttatgacaatgactatgtcggctggggacgaactgcagaagatgcatggaaatatgaccgcgacctgaagcatattgcagggcaatttatctggaccggctttgattatattggcgagccgacgccatattataattcctatcctgcaaaaagctcctattttggtgctgtggatacggctggttttccaaaggatattttctactattaccaaagccaatggaaaaaggagcctatggtccacctgctgccgcattggaactggaaggaaggggaaaaggtccgcgtcttagcttataccaatgcaagtaaggttgaacttgttctaaatggtgaatcgttaggggagaagaactatgacaacaaacaaacctcctggggagcaccatacaaagaaacaaaggatggaaaaacctatttggagtgggccgtaccatttaaaccgggcaaattagaagccgtcgccaaggatgaaaacggcaaagtgatcgcccgcgatcaggtagtgaccgctggtgagccagcctctgtcagattaacggctgatcgtaaggtggtcaaggcggacggtacggatctgtcgtttattacagcagacattgttgatagtaaagggattgttgtcccggatgccgatcatctgattacatttaacgtaacgggccaaggggaattggccggggttgataacggaaacgcgtccagtgtggagcgttacaaggacaacaagcgcaaggctttcagcgggaaagcattggcgattgttcaatcaagtaagctttctggaaaaattacggtccatgcgtcagtggcagggctttcgagcgattccacgagcgtatttacggtaacgccagctgaccatgacaaaaagattgtagctgggattgatgatgttaaccttactgtcgatgtcaatgaagcaccaaagcttccttcagaaatcaaggtttattacagtgatgagagtgcagctgcgaagaatgtgacttgggatgaggtggatccaaagcagtacagcactgttggtgaattcacagtggaaggcagtgtcgagggaacttcgctgaaggcaaaggcatttgttattgtcaaaggaattgtcgccgtcaagccttattcaacggcaacaaaggttggtgtacagccggtgctgcctgaaaaagcaacccttctttacagtgatggaacaaccaagggagcaactgtcacgtgggatgagatccctgaggacaagctggcaaaagagggccggtttaccgtcgagggcagtgtggagggaacagacctcaaggctaatgtctatgtcagggtgacaaatgaagtaaaatcagtgaatattatgcttcaggagcagggttcagcttatccaaagctcgaagctacttttaccaatccagctgacaatcttcagcatttgaacgatggcatcaagagctataccaataacccggtcaaccgctggacgaactggacaagaacaccgcgtgatgctggtgactcgattacagttaattttggcaagaagcatgtgattaataatctagatttatttgtttttaccgacagcggcacggtggttccagaaaaggcagaggtccaatattgggatggaacggcgtggaaggatgtcgaaaatctaacacagccatcgccatatgtggtagagaaaaatgaacttacatttgatgcggtcgcgacagaaaagctgaaattccatttgacaccatctgtgaaagggaaattcctagctctaacggaagcagaggtgtacgccgatcagattgtgatgggtgaaacagcaaaacttcaaagtattacggtgaatgggaaagcattagaaggctttgatcacgctaaaaagaattatgaacttgtacttccatatggaagcgagcttcctaagattgaggcggctgctgccgacaatgcaactgtcaccattttaccggcattctcctatccgggaacagcaaaactatttgtcacttcagaggatgggaaggtaactactgagtacagtattggtgtttctacagaagagccaaagctcgtctccgca

SEQ ID NO: 8 - DNA, 2541 bp, Bacillus circulans
  source 1..2541: mol_type = genomic DNA
gtgaaaaaagcgattagctgcgtttttttaatttcagcactgattctatcaagctttcaagtccctgtacagggacaagccatgtcaaaaacgacatcggcagcaggaaacagtgtgagctatgatggagagagacgagtgaattttaacgagaattggcgatttcaacgagaaaccaatggaagtattgccggagcacagaatcctggctttgacgattcctcctggcggaaattaaatctgccgcatgactggagtattgaattagattttaataaaaattctcttgccacacatgaaggcggttatttggacggcggaatcggctggtaccgaaaaacctttacaatcccggaatcgatgaagggaaaacgaatttcgcttgattttgatggcgtttacatgaacagcaccacctatctaaacggggaagtgctcgggacctatccgtttggttataatgccttttcctatgatatttccgacaaactttataaagatggcagggcgaatgtccttgttgtcaaagtcaataacacccagccgagcagccgctggtattcggggagcgggatctaccggaatgtctatctcactgtgaccgatcccatccatgtggctcgctacggaacatttgtgacaacacccaatttagagaaatcgataaaagaagacagggctgatgtgaacatcaagacgaaaatcagtaacgatgctgctgaggcgaaacaggtaaagattaaatcaaccatctacgatggggctgggaacaccgtacagacagtggaaacggaggaaaaaacagctgccgccggcacggtgactccgttcgaacaaaacacagtcatcaagcagccgaagctttggagcattgacaagccttatcgatataaccttgttacagaagtcatcgttggcgggcaaacggtggatacgtatgaaacaaaatttggtgtcaggtatttcaaatttgatgaaaacgaaggcttttccttaaatggagagtatatgaagctgcacggcgtttcgatgcaccatgatttaggggcgcttggggcggcaacgaatgcacgcggcgtggaaagacaaatgcagattatgaaggatatgggggtcaatgccatcagggttacccacaacccggcatcaccggaactgctggaggcagctaataaattagggctattcatcatcgaggaggcatttgacagctgggcccagtcaaagaaaccctatgactatggccgttttttcaatgcatgggctgagcacgacattaaggaaatggtcgatcggggcaaaaacgaaccagctattatcatgtggtcgatcggaaatgaaatatatgatacgaccaatgccgctggtgtggaaacagcacgaaatttagtgggttgggtaaaagaaattgacaccacaaggccgacaacgatcggcgaggataaaacccgcggagacaaagtaaatgttacacctatcaacagctacatcaaggagatttttaatattgtcgatgtggtcggactgaactacagcgagaacaactatgatggctaccacaagcagaatccgtcatggaagctgtacggctcggagacgtcctcggcaacccgttcgcgtggtgtctacacgcatccgtaccagtataaccaaagcacaaagtatgctgatttacagcaatcctcttatgacaatgactatgtcggctggggacgaactgcagaagatgcatggaaatatgaccgcgacctgaagcatattgcagggcaatttatctggaccggctttgattatattggcgagccgacgccatattataattcctatcctgcaaaaagctcctattttggtgctgtggatacggctggttttccaaaggatattttctactattaccaaagccaatggaaaaaggagcctatggtccacctgctgccgcattggaactggaaggaaggggaaaaggtccgcgtcttagcttataccaatgcaagtaaggttgaacttgttctaaatggtgaatcgttaggggagaagaactatgacaacaaacaaacctcctggggagcaccatacaaagaaacaaaggatggaaaaacctatttggagtgggccgtaccatttaaaccgggcaaattagaagccgtcgccaaggatgaaaacggcaaagtgatcgcccgcgatcaggtagtgaccgctggtgagccagcctctgtcagattaacggctgatcgtaaggtggtcaaggcggacggtacggatctgtcgtttattacagcagacattgttgatagtaaagggattgttgtcccggatgccgatcatctgattacatttaacgtaacgggccaaggggaattggccggggttgataacggaaacgcgtccagtgtggagcgttacaaggacaacaagcgcaaggctttcagcgggaaagcattggcgattgttcaatcaagtaagctttctggaaaaattacggtccatgcgtcagtggcagggctttcgagcgattccacgagcgtatttacggtaacgcca

SEQ ID NO: 9 - protein, 4 aa, synthetic construct
  REGION 1..4: note = sequence of mutated position
NFFN

SEQ ID NO: 10 - protein, 4 aa, synthetic construct
  REGION 1..4: note = sequence of mutated position
NWWN

SEQ ID NO: 11 - protein, 4 aa, synthetic construct
  REGION 1..4: note = sequence of mutated position
PWWY

SEQ ID NO: 12 - protein, 6 aa, synthetic construct
  REGION 1..6: note = sequence of mutated position
PAAAAY

SEQ ID NO: 13 - protein, 6 aa, synthetic construct
  REGION 1..6: note = sequence of mutated position
PFFFFY

SEQ ID NO: 14 - protein, 4 aa, synthetic construct
  REGION 1..4: note = sequence of mutated position
RAAG

SEQ ID NO: 15 - protein, 4 aa, synthetic construct
  REGION 1..4: note = sequence of mutated position
RFFG

SEQ ID NO: 16 - protein, 4 aa, synthetic construct
  REGION 1..4: note = sequence of mutated position
RKKG

SEQ ID NO: 17 - protein, 4 aa, synthetic construct
  REGION 1..4: note = sequence of mutated position
RPPG

SEQ ID NO: 18 - protein, 4 aa, synthetic construct
  REGION 1..4: note = sequence of mutated position
RRRG

SEQ ID NO: 19 - protein, 4 aa, synthetic construct
  REGION 1..4: note = sequence of mutated position
RSSG

SEQ ID NO: 20 - protein, 4 aa, synthetic construct
  REGION 1..4: note = sequence of mutated position
RWWG

SEQ ID NO: 21 - protein, 5 aa, synthetic construct
  REGION 1..5: note = sequence of mutated position
GSSSD

SEQ ID NO: 22 - protein, 6 aa, synthetic construct
  REGION 1..6: note = sequence of mutated position
RAAAAG

SEQ ID NO: 23 - protein, 6 aa, synthetic construct
  REGION 1..6: note = sequence of mutated position
RDDDDG

SEQ ID NO: 24 - protein, 6 aa, synthetic construct
  REGION 1..6: note = sequence of mutated position
RFFFFG

SEQ ID NO: 25 - protein, 6 aa, synthetic construct
  REGION 1..6: note = sequence of mutated position
RPPPPG

SEQ ID NO: 26 - protein, 6 aa, synthetic construct
  REGION 1..6: note = sequence of mutated position
RRRRRG

SEQ ID NO: 27 - protein, 6 aa, synthetic construct
  REGION 1..6: note = sequence of mutated position
RSSSSG

SEQ ID NO: 28 - protein, 6 aa, synthetic construct
  REGION 1..6: note = sequence of mutated position
RWWWWG

SEQ ID NO: 29 - protein, 10 aa, synthetic construct
  REGION 1..10: note = sequence of mutated position
RAAAAAAAAG

SEQ ID NO: 30 - protein, 10 aa, synthetic construct
  REGION 1..10: note = sequence of mutated position
RDDDDDDDDG

SEQ ID NO: 31 - protein, 10 aa, synthetic construct
  REGION 1..10: note = sequence of mutated position
RFFFFFFFFG

SEQ ID NO: 32 - protein, 10 aa, synthetic construct
  REGION 1..10: note = sequence of mutated position
RKKKKKKKKG

SEQ ID NO: 33 - protein, 10 aa, synthetic construct
  REGION 1..10: note = sequence of mutated position
RPPPPPPPPG